European Patent Application EP 4 733 411 A1, published April 29, 2026. Title: 核酸増幅における増幅バイアスの低減方法. Applicant: 東洋紡株式会社. The sequence listing filed with the application follows.

SEQUENCE LISTING (28 sequences)

SEQ ID NO: 1 - protein, 249 aa, Thermococcus kodakaraensis
MPFEVVFDGAKEFADLIATASNLIDEAAFKFTEEGISMRAMDPSRVVLIDLNLPESIFSKYEVEEPETIGINMDQFKKILKRGKAKDTLILRKGDENFLEITFEGTAKRTFRLPLIDVEELELELPELPFTAKVVLLGEVLKEGIKDASLVSDAIKFIAKENEFTMKAEGETNEVEIRLTLEDEGLLDLEVEEETKSAYGIRYLSDMVKGIGKADEVILRFGNEMPLQMEYMIRDEGRLTFLLAPRVEE

SEQ ID NO: 2 - protein, 249 aa, Pyrococcus furiosus
MPFEIVFEGAKEFAQLIDTASKLIDEAAFKVTEDGISMRAMDPSRVVLIDLNLPSSIFSKYEVVEPETIGVNMDHLKKILKRGKAKDTLILKKGEENFLEITIQGTATRTFRVPLIDVEEMEVDLPELPFTAKVVVLGEVLKDAVKDASLVSDSIKFIARENEFIMKAEGETQEVEIKLTLEDEGLLDIEVQEETKSAYGVSYLSDMVKGLGKADEVTIKFGNEMPMQMEYYIRDEGRLTFLLAPRVEE

SEQ ID NO: 3 - DNA, 750 bp, Thermococcus kodakaraensis
  source 1..750: mol_type = genomic DNA
atgccgttcgaagttgtttttgacggggccaaggagtttgcagacctgatagcgaccgcaagcaacctcatcgacgaggccgcctttaagttcactgaggaaggcataagcatgcgcgcaatggacccgagcagggtcgttctcattgacctcaacctgcccgaaagcatcttctccaagtacgaggtcgaagagcccgagacaatcggcatcaacatggaccagttcaagaaaatcctcaagcgcggcaaggcgaaagacaccctcatactcaggaagggcgacgagaacttccttgagataacttttgagggaaccgccaagaggacattcaggctccctctgatagatgtggaagagcttgagctggagcttcccgagctcccgttcacggctaaggtagtcctcctcggtgaggttctcaaggagggcataaaggacgcttccctcgtcagcgacgccatcaagttcatagcaaaggagaacgagttcacaatgaaggccgagggcgagaccaacgaggtcgagataaggcttacccttgaggacgagggccttctcgaccttgaagtcgaggaagagaccaagagtgcctacggcataagatacctcagcgacatggtcaagggcatcgggaaggccgacgaagttatcctccgcttcggcaacgagatgccgctccagatggagtacatgatcagagacgagggcagactgaccttcctgctcgctccgcgcgttgaggagtga

SEQ ID NO: 4 - DNA, 750 bp, Pyrococcus furiosus
  source 1..750: mol_type = genomic DNA
atgccatttgaaatcgtatttgaaggtgcaaaagagtttgcccaacttatagacaccgcaagtaagttaatagatgaggccgcgtttaaagttacagaagatgggataagcatgagggccatggatccaagtagagttgtcctgattgacctaaatctcccgtcaagcatatttagcaaatatgaagttgttgaaccagaaacaattggagttaacatggaccacctaaagaagatcctaaagagaggtaaagcaaaggacaccttaatactcaagaaaggagaggaaaacttcttagagataacaattcaaggaactgcaacaagaacatttagagttcccctaatagatgtagaagagatggaagttgacctcccagaacttccattcactgcaaaggttgtagttcttggagaagtcctaaaagatgctgttaaagatgcctctctagtgagtgacagcataaaatttattgccagggaaaatgaatttataatgaaggcagagggagaaacccaggaagttgagataaagctaactcttgaagatgagggattattggacatcgaggttcaagaggagacaaagagcgcatatggagtcagctatctctccgacatggttaaaggacttggaaaggccgatgaagttacaataaagtttggaaatgaaatgcccatgcaaatggagtattacattagagatgaaggaagacttacattcctactggctccaagagttgaagagtga

SEQ ID NO: 5 - DNA, 22 bp, Artificial sequence primer
  misc_feature 1..22: note = Artificial sequence primer
  source 1..22: mol_type = other DNA
ttaggccttagcgggcttagac

SEQ ID NO: 6 - DNA, 22 bp, Artificial sequence primer
  misc_feature 1..22: note = Artificial sequence primer
  source 1..22: mol_type = other DNA
ccaggatttttgatgggacacg

SEQ ID NO: 7 - DNA, 24 bp, Artificial sequence primer
  misc_feature 1..24: note = Artificial sequence primer
  source 1..24: mol_type = other DNA
aatgatacggcgaccaccgagatc

SEQ ID NO: 8 - DNA, 22 bp, Artificial sequence primer
  misc_feature 1..22: note = Artificial sequence primer
  source 1..22: mol_type = other DNA
caagcagaagacggcatacgag

SEQ ID NO: 9 - protein, 249 aa, Thermococcus kodakaraensis
MPFEVVFDGAKEFADLIATASNLIDEAAFKFTEEGISMRAMDPSRVVLIDLNLPESIFSKYEVEEPETIGINLDQFKKILKRGKAKDTLILRKGDENFLEITFEGTAKRTFRLPLIDVEELELELPELPFTAKVVLLGEVLKEGIKDASLVSDAIKFIAKENEFTMKAEGETNEVEIRLTLEDEGLLDLEVEEETKSAYGIRYLSDMVKGIGKADEVILRFGNEMPLQMEYMIRDEGRLTFLLAPRVEE

SEQ ID NO: 10 - DNA, 750 bp, Thermococcus kodakaraensis
  source 1..750: mol_type = other DNA
atgccgttcgaagttgtttttgacggggccaaggagtttgcagacctgatagcgaccgcaagcaacctcatcgacgaggccgcctttaagttcactgaggaaggcataagcatgcgcgcaatggacccgagcagggtcgttctcattgacctcaacctgcccgaaagcatcttctccaagtacgaggtcgaagagcccgagacaatcggcatcaacctggaccagttcaagaaaatcctcaagcgcggcaaggcgaaagacaccctcatactcaggaagggcgacgagaacttccttgagataacttttgagggaaccgccaagaggacattcaggctccctctgatagatgtggaagagcttgagctggagcttcccgagctcccgttcacggctaaggtagtcctcctcggtgaggttctcaaggagggcataaaggacgcttccctcgtcagcgacgccatcaagttcatagcaaaggagaacgagttcacaatgaaggccgagggcgagaccaacgaggtcgagataaggcttacccttgaggacgagggccttctcgaccttgaagtcgaggaagagaccaagagtgcctacggcataagatacctcagcgacatggtcaagggcatcgggaaggccgacgaagttatcctccgcttcggcaacgagatgccgctccagatggagtacatgatcagagacgagggcagactgaccttcctgctcgctccgcgcgttgaggagtga

SEQ ID NO: 11 - protein, 249 aa, Thermococcus kodakaraensis
MPFEVVFDGAKEFADLIATASNLIDEAAFKFTEEGISMRAMDPSRVVLIDLNLPESIFSKYEVEEPETIGINLDQFKKILKRGKAKDTLILRKGDENFLEITFEGTAKRTFRLPLIDVEELELELPELPFTAKVVLLGEVLKRGIKDASLVSDAIKFIAKENEFTMKAEGETNEVEIRLTLEDEGLLDLEVEEETKSAYGIRYLSDMVKGIGKADEVILRFGNEMPLQMEYMIRDEGRLTFLLAPRVEE

SEQ ID NO: 12 - DNA, 750 bp, Thermococcus kodakaraensis
  source 1..750: mol_type = other DNA
atgccgttcgaagttgtttttgacggggccaaggagtttgcagacctgatagcgaccgcaagcaacctcatcgacgaggccgcctttaagttcactgaggaaggcataagcatgcgcgcaatggacccgagcagggtcgttctcattgacctcaacctgcccgaaagcatcttctccaagtacgaggtcgaagagcccgagacaatcggcatcaacctggaccagttcaagaaaatcctcaagcgcggcaaggcgaaagacaccctcatactcaggaagggcgacgagaacttccttgagataacttttgagggaaccgccaagaggacattcaggctccctctgatagatgtggaagagcttgagctggagcttcccgagctcccgttcacggctaaggtagtcctcctcggtgaggttctcaagcgtggcataaaggacgcttccctcgtcagcgacgccatcaagttcatagcaaaggagaacgagttcacaatgaaggccgagggcgagaccaacgaggtcgagataaggcttacccttgaggacgagggccttctcgaccttgaagtcgaggaagagaccaagagtgcctacggcataagatacctcagcgacatggtcaagggcatcgggaaggccgacgaagttatcctccgcttcggcaacgagatgccgctccagatggagtacatgatcagagacgagggcagactgaccttcctgctcgctccgcgcgttgaggagtga

SEQ ID NO: 13 - protein, 249 aa, Thermococcus kodakaraensis
MPFEVVFDGAKEFADLIATASNLIDEAAFKFTEEGISMRAMDPSRVVLIDLNLPESIFSKYEVEEPETIGINLDQFKKILKRGKAKDTLILRKGDENFLEITFEGTAKRTFRLPLIDVEELELELPELPFTAKVVLLGEVLKKGIKDASLVSDAIKFIAKENEFTMKAEGETNEVEIRLTLEDEGLLDLEVEEETKSAYGIRYLSDMVKGIGKADEVILRFGNEMPLQMEYMIRDEGRLTFLLAPRVEE

SEQ ID NO: 14 - DNA, 750 bp, Thermococcus kodakaraensis
  source 1..750: mol_type = other DNA
atgccgttcgaagttgtttttgacggggccaaggagtttgcagacctgatagcgaccgcaagcaacctcatcgacgaggccgcctttaagttcactgaggaaggcataagcatgcgcgcaatggacccgagcagggtcgttctcattgacctcaacctgcccgaaagcatcttctccaagtacgaggtcgaagagcccgagacaatcggcatcaacctggaccagttcaagaaaatcctcaagcgcggcaaggcgaaagacaccctcatactcaggaagggcgacgagaacttccttgagataacttttgagggaaccgccaagaggacattcaggctccctctgatagatgtggaagagcttgagctggagcttcccgagctcccgttcacggctaaggtagtcctcctcggtgaggttctcaagaaaggcataaaggacgcttccctcgtcagcgacgccatcaagttcatagcaaaggagaacgagttcacaatgaaggccgagggcgagaccaacgaggtcgagataaggcttacccttgaggacgagggccttctcgaccttgaagtcgaggaagagaccaagagtgcctacggcataagatacctcagcgacatggtcaagggcatcgggaaggccgacgaagttatcctccgcttcggcaacgagatgccgctccagatggagtacatgatcagagacgagggcagactgaccttcctgctcgctccgcgcgttgaggagtga

SEQ ID NO: 15 - protein, 249 aa, Thermococcus kodakaraensis
MPFEVVFDGAKEFADLIATASNLIDEAAFKFTEEGISMRAMDPSRVVLIDLNLPESIFSKYEVEEPETIGINLDQFKKILKRGKAKDTLILRKGDENFLEITFEGTAKRTFRLPLIDVEELELELPELPFTAKVVLLGEVLKEGIKAASLVSDAIKFIAKENEFTMKAEGETNEVEIRLTLEDEGLLDLEVEEETKSAYGIRYLSDMVKGIGKADEVILRFGNEMPLQMEYMIRDEGRLTFLLAPRVEE

SEQ ID NO: 16 - DNA, 750 bp, Thermococcus kodakaraensis
  source 1..750: mol_type = other DNA
atgccgttcgaagttgtttttgacggggccaaggagtttgcagacctgatagcgaccgcaagcaacctcatcgacgaggccgcctttaagttcactgaggaaggcataagcatgcgcgcaatggacccgagcagggtcgttctcattgacctcaacctgcccgaaagcatcttctccaagtacgaggtcgaagagcccgagacaatcggcatcaacctggaccagttcaagaaaatcctcaagcgcggcaaggcgaaagacaccctcatactcaggaagggcgacgagaacttccttgagataacttttgagggaaccgccaagaggacattcaggctccctctgatagatgtggaagagcttgagctggagcttcccgagctcccgttcacggctaaggtagtcctcctcggtgaggttctcaaggagggcataaaggccgcttccctcgtcagcgacgccatcaagttcatagcaaaggagaacgagttcacaatgaaggccgagggcgagaccaacgaggtcgagataaggcttacccttgaggacgagggccttctcgaccttgaagtcgaggaagagaccaagagtgcctacggcataagatacctcagcgacatggtcaagggcatcgggaaggccgacgaagttatcctccgcttcggcaacgagatgccgctccagatggagtacatgatcagagacgagggcagactgaccttcctgctcgctccgcgcgttgaggagtga

SEQ ID NO: 17 - protein, 249 aa, Thermococcus kodakaraensis
MPFEVVFDGAKEFADLIATASNLIDEAAFKFTEEGISMRAMDPSRVVLIDLNLPESIFSKYEVEEPETIGINLDQFKKILKRGKAKDTLILRKGDENFLEITFEGTAKRTFRLPLIDVEELELELPELPFTAKVVLLGEVLKEGIKGASLVSDAIKFIAKENEFTMKAEGETNEVEIRLTLEDEGLLDLEVEEETKSAYGIRYLSDMVKGIGKADEVILRFGNEMPLQMEYMIRDEGRLTFLLAPRVEE

SEQ ID NO: 18 - DNA, 750 bp, Thermococcus kodakaraensis
  source 1..750: mol_type = other DNA
atgccgttcgaagttgtttttgacggggccaaggagtttgcagacctgatagcgaccgcaagcaacctcatcgacgaggccgcctttaagttcactgaggaaggcataagcatgcgcgcaatggacccgagcagggtcgttctcattgacctcaacctgcccgaaagcatcttctccaagtacgaggtcgaagagcccgagacaatcggcatcaacctggaccagttcaagaaaatcctcaagcgcggcaaggcgaaagacaccctcatactcaggaagggcgacgagaacttccttgagataacttttgagggaaccgccaagaggacattcaggctccctctgatagatgtggaagagcttgagctggagcttcccgagctcccgttcacggctaaggtagtcctcctcggtgaggttctcaaggagggcataaagggtgcttccctcgtcagcgacgccatcaagttcatagcaaaggagaacgagttcacaatgaaggccgagggcgagaccaacgaggtcgagataaggcttacccttgaggacgagggccttctcgaccttgaagtcgaggaagagaccaagagtgcctacggcataagatacctcagcgacatggtcaagggcatcgggaaggccgacgaagttatcctccgcttcggcaacgagatgccgctccagatggagtacatgatcagagacgagggcagactgaccttcctgctcgctccgcgcgttgaggagtga

SEQ ID NO: 19 - protein, 249 aa, Pyrococcus furiosus
MPFEIVFEGAKEFAQLIDTASKLIDEAAFKVTEDGISMRAMDPSRVVLIDLNLPSSIFSKYEVVEPETIGVNLDHLKKILKRGKAKDTLILKKGEENFLEITIQGTATRTFRVPLIDVEEMEVDLPELPFTAKVVVLGEVLKDAVKDASLVSDSIKFIARENEFIMKAEGETQEVEIKLTLEDEGLLDIEVQEETKSAYGVSYLSDMVKGLGKADEVTIKFGNEMPMQMEYYIRDEGRLTFLLAPRVEE

SEQ ID NO: 20 - DNA, 750 bp, Pyrococcus furiosus
  source 1..750: mol_type = other DNA
atgccatttgaaatcgtatttgaaggtgcaaaagagtttgcccaacttatagacaccgcaagtaagttaatagatgaggccgcgtttaaagttacagaagatgggataagcatgagggccatggatccaagtagagttgtcctgattgacctaaatctcccgtcaagcatatttagcaaatatgaagttgttgaaccagaaacaattggagttaacctggaccacctaaagaagatcctaaagagaggtaaagcaaaggacaccttaatactcaagaaaggagaggaaaacttcttagagataacaattcaaggaactgcaacaagaacatttagagttcccctaatagatgtagaagagatggaagttgacctcccagaacttccattcactgcaaaggttgtagttcttggagaagtcctaaaagatgctgttaaagatgcctctctagtgagtgacagcataaaatttattgccagggaaaatgaatttataatgaaggcagagggagaaacccaggaagttgagataaagctaactcttgaagatgagggattattggacatcgaggttcaagaggagacaaagagcgcatatggagtcagctatctctccgacatggttaaaggacttggaaaggccgatgaagttacaataaagtttggaaatgaaatgcccatgcaaatggagtattacattagagatgaaggaagacttacattcctactggctccaagagttgaagagtga

SEQ ID NO: 21 - protein, 249 aa, Pyrococcus furiosus
MPFEIVFEGAKEFAQLIDTASKLIDEAAFKVTEDGISMRAMDPSRVVLIDLNLPSSIFSKYEVVEPETIGVNLDHLKKILKRGKAKDTLILKKGEENFLEITIQGTATRTFRVPLIDVEEMEVDLPELPFTAKVVVLGEVLKRAVKDASLVSDSIKFIARENEFIMKAEGETQEVEIKLTLEDEGLLDIEVQEETKSAYGVSYLSDMVKGLGKADEVTIKFGNEMPMQMEYYIRDEGRLTFLLAPRVEE

SEQ ID NO: 22 - DNA, 750 bp, Pyrococcus furiosus
  source 1..750: mol_type = other DNA
atgccatttgaaatcgtatttgaaggtgcaaaagagtttgcccaacttatagacaccgcaagtaagttaatagatgaggccgcgtttaaagttacagaagatgggataagcatgagggccatggatccaagtagagttgtcctgattgacctaaatctcccgtcaagcatatttagcaaatatgaagttgttgaaccagaaacaattggagttaacctggaccacctaaagaagatcctaaagagaggtaaagcaaaggacaccttaatactcaagaaaggagaggaaaacttcttagagataacaattcaaggaactgcaacaagaacatttagagttcccctaatagatgtagaagagatggaagttgacctcccagaacttccattcactgcaaaggttgtagttcttggagaagtcctaaaacgtgctgttaaagatgcctctctagtgagtgacagcataaaatttattgccagggaaaatgaatttataatgaaggcagagggagaaacccaggaagttgagataaagctaactcttgaagatgagggattattggacatcgaggttcaagaggagacaaagagcgcatatggagtcagctatctctccgacatggttaaaggacttggaaaggccgatgaagttacaataaagtttggaaatgaaatgcccatgcaaatggagtattacattagagatgaaggaagacttacattcctactggctccaagagttgaagagtga

SEQ ID NO: 23 - protein, 249 aa, Pyrococcus furiosus
MPFEIVFEGAKEFAQLIDTASKLIDEAAFKVTEDGISMRAMDPSRVVLIDLNLPSSIFSKYEVVEPETIGVNLDHLKKILKRGKAKDTLILKKGEENFLEITIQGTATRTFRVPLIDVEEMEVDLPELPFTAKVVVLGEVLKKAVKDASLVSDSIKFIARENEFIMKAEGETQEVEIKLTLEDEGLLDIEVQEETKSAYGVSYLSDMVKGLGKADEVTIKFGNEMPMQMEYYIRDEGRLTFLLAPRVEE

SEQ ID NO: 24 - DNA, 750 bp, Pyrococcus furiosus
  source 1..750: mol_type = other DNA
atgccatttgaaatcgtatttgaaggtgcaaaagagtttgcccaacttatagacaccgcaagtaagttaatagatgaggccgcgtttaaagttacagaagatgggataagcatgagggccatggatccaagtagagttgtcctgattgacctaaatctcccgtcaagcatatttagcaaatatgaagttgttgaaccagaaacaattggagttaacctggaccacctaaagaagatcctaaagagaggtaaagcaaaggacaccttaatactcaagaaaggagaggaaaacttcttagagataacaattcaaggaactgcaacaagaacatttagagttcccctaatagatgtagaagagatggaagttgacctcccagaacttccattcactgcaaaggttgtagttcttggagaagtcctaaaaaaagctgttaaagatgcctctctagtgagtgacagcataaaatttattgccagggaaaatgaatttataatgaaggcagagggagaaacccaggaagttgagataaagctaactcttgaagatgagggattattggacatcgaggttcaagaggagacaaagagcgcatatggagtcagctatctctccgacatggttaaaggacttggaaaggccgatgaagttacaataaagtttggaaatgaaatgcccatgcaaatggagtattacattagagatgaaggaagacttacattcctactggctccaagagttgaagagtga

SEQ ID NO: 25 - protein, 249 aa, Pyrococcus furiosus
MPFEIVFEGAKEFAQLIDTASKLIDEAAFKVTEDGISMRAMDPSRVVLIDLNLPSSIFSKYEVVEPETIGVNLDHLKKILKRGKAKDTLILKKGEENFLEITIQGTATRTFRVPLIDVEEMEVDLPELPFTAKVVVLGEVLKDAVKAASLVSDSIKFIARENEFIMKAEGETQEVEIKLTLEDEGLLDIEVQEETKSAYGVSYLSDMVKGLGKADEVTIKFGNEMPMQMEYYIRDEGRLTFLLAPRVEE

SEQ ID NO: 26 - DNA, 750 bp, Pyrococcus furiosus
  source 1..750: mol_type = other DNA
atgccatttgaaatcgtatttgaaggtgcaaaagagtttgcccaacttatagacaccgcaagtaagttaatagatgaggccgcgtttaaagttacagaagatgggataagcatgagggccatggatccaagtagagttgtcctgattgacctaaatctcccgtcaagcatatttagcaaatatgaagttgttgaaccagaaacaattggagttaacctggaccacctaaagaagatcctaaagagaggtaaagcaaaggacaccttaatactcaagaaaggagaggaaaacttcttagagataacaattcaaggaactgcaacaagaacatttagagttcccctaatagatgtagaagagatggaagttgacctcccagaacttccattcactgcaaaggttgtagttcttggagaagtcctaaaagatgctgttaaagccgcctctctagtgagtgacagcataaaatttattgccagggaaaatgaatttataatgaaggcagagggagaaacccaggaagttgagataaagctaactcttgaagatgagggattattggacatcgaggttcaagaggagacaaagagcgcatatggagtcagctatctctccgacatggttaaaggacttggaaaggccgatgaagttacaataaagtttggaaatgaaatgcccatgcaaatggagtattacattagagatgaaggaagacttacattcctactggctccaagagttgaagagtga

SEQ ID NO: 27 - protein, 249 aa, Pyrococcus furiosus
MPFEIVFEGAKEFAQLIDTASKLIDEAAFKVTEDGISMRAMDPSRVVLIDLNLPSSIFSKYEVVEPETIGVNLDHLKKILKRGKAKDTLILKKGEENFLEITIQGTATRTFRVPLIDVEEMEVDLPELPFTAKVVVLGEVLKDAVKGASLVSDSIKFIARENEFIMKAEGETQEVEIKLTLEDEGLLDIEVQEETKSAYGVSYLSDMVKGLGKADEVTIKFGNEMPMQMEYYIRDEGRLTFLLAPRVEE

SEQ ID NO: 28 - DNA, 750 bp, Pyrococcus furiosus
  source 1..750: mol_type = other DNA
atgccatttgaaatcgtatttgaaggtgcaaaagagtttgcccaacttatagacaccgcaagtaagttaatagatgaggccgcgtttaaagttacagaagatgggataagcatgagggccatggatccaagtagagttgtcctgattgacctaaatctcccgtcaagcatatttagcaaatatgaagttgttgaaccagaaacaattggagttaacctggaccacctaaagaagatcctaaagagaggtaaagcaaaggacaccttaatactcaagaaaggagaggaaaacttcttagagataacaattcaaggaactgcaacaagaacatttagagttcccctaatagatgtagaagagatggaagttgacctcccagaacttccattcactgcaaaggttgtagttcttggagaagtcctaaaagatgctgttaaaggtgcctctctagtgagtgacagcataaaatttattgccagggaaaatgaatttataatgaaggcagagggagaaacccaggaagttgagataaagctaactcttgaagatgagggattattggacatcgaggttcaagaggagacaaagagcgcatatggagtcagctatctctccgacatggttaaaggacttggaaaggccgatgaagttacaataaagtttggaaatgaaatgcccatgcaaatggagtattacattagagatgaaggaagacttacattcctactggctccaagagttgaagagtga